European Patent Specification EP 4 069 278 B1, published June 11, 2025. Title: METHODS AND COMPOSITIONS FOR THE TREATMENT AND PREVENTION OF TYPE 1 DIABETES. Applicant: DR. MARY MORRIS & ASSOCIATES, LLC. The sequence listing filed with the application follows.

SEQUENCE LISTING (24 sequences)

SEQ ID NO: 1 - protein, 30 aa, Homo sapiens
FVNQHLCGSHLVEALYLVCGERGFFYTPKT

SEQ ID NO: 2 - protein, 21 aa, Homo sapiens
GIVEQCCTSICSLYQLENYCN

SEQ ID NO: 3 - protein, 21 aa, Homo sapiens
LCGSHLVEALYLVCGERGFFY

SEQ ID NO: 4 - protein, 15 aa, Homo sapiens
CCTSICSLYQLENYC

SEQ ID NO: 5 - protein, 20 aa, Homo sapiens
GIVEQCCTSICSLYQLENYC

SEQ ID NO: 6 - protein, 17 aa, Homo sapiens
EQCCTSICSLYQLENYC

SEQ ID NO: 7 - protein, 24 aa, Homo sapiens
NQHLCGSHLVEALYLVCGERGFFY

SEQ ID NO: 8 - protein, 24 aa, Homo sapiens
QHLCGSHLVEALYLVCGERGFFYT

SEQ ID NO: 9 - protein, 20 aa, Homo sapiens
CGSHLVEALYLVCGERGFFY

SEQ ID NO: 10 - protein, 86 aa, Homo sapiens
FVNQHLCGSHLVEALYLVCGERGFFYTPKTRREAEDLQVGQVELGGGPGAGSLQPLALEGSLQKRGIVEQCCTSICSLYQLENYCN

SEQ ID NO: 11 - protein, 86 aa, Unknown; identical to SEQ ID NO: 10
  Description of Unknown: Great ape insulin sequence

SEQ ID NO: 12 - protein, 86 aa, Macaca fascicularis
FVNQHLCGSHLVEALYLVCGERGFFYTPKTRREAEDPQVGQVELGGGPGAGSLQPLALEGSLQKRGIVEQCCTSICSLYQLENYCN

SEQ ID NO: 13 - protein, 86 aa, Unknown
  Description of Unknown: Rabbit insulin sequence
FVNQHLCGSHLVEALYLVCGERGFFYTPKSRREVEELQVGQAELGGGPGAGGLQPSALELALQKRGIVEQCCTSICSLYQLENYCN

SEQ ID NO: 14 - protein, 86 aa, Canis sp.
FVNQHLCGSHLVEALYLVCGERGFFYTPKARREVEDLQVRDVELAGAPGEGGLQPLALEGALQKRGIVEQCCTSICSLYQLENYCN

SEQ ID NO: 15 - protein, 86 aa, Equus sp.
  MOD_RES (31)..(32): Any amino acid
  MOD_RES (64)..(65): Any amino acid
FVNQHLCGSHLVEALYLVCGERGFFYTPKAXXEAEDPQVGEVELGGGPGLGGLQPLALAGPQQXXGIVEQCCTGICSLYQLENYCN

SEQ ID NO: 16 - protein, 84 aa, Sus scrofa
FVNQHLCGSHLVEALYLVCGERGFFYTPKARREAENPQAGAVELGGGLGGLQALALEGPPQKRGIVEQCCTSICSLYQLENYCN

SEQ ID NO: 17 - protein, 86 aa, Unknown
  Description of Unknown: Hamster insulin sequence
FVNQHLCGSHLVEALYLVCGERGFFYTPKSRRGVEDPQVAQLELGGGPGADDLQTLALEVAQQKRGIVDQCCTSICSLYQLENYCN

SEQ ID NO: 18 - protein, 86 aa, Rattus sp.
FVKQHLCGSHLVEALYLVCGERGFFYTPMSRREVEDPQVAQLELGGGPGAGDLQTLALEVARQKRGIVDQCCTSICSLYQLENYCN

SEQ ID NO: 19 - protein, 86 aa, Mus sp.
FVKQHLCGSHLVEALYLVCGERGFFYTPMSRREVEDPQVAQLELGGGPGAGDLQTLALEVAQQKRGIVDQCCTSICSLYQLENYCN

SEQ ID NO: 20 - protein, 86 aa, Felis sp.
FVNQHLCGSHLVEALYLVCGERGFFYTPKARREAEDLQGKDAELGEAPGAGGLQPSALEAPLQKRGIVEQCCASVCSLYQLEHYCN

SEQ ID NO: 21 - protein, 86 aa, Rattus sp.
FVKQHLCGPHLVEALYLVCGERGFFYTPKSRREVEDPQVPQLELGGGPEAGDLQTLALEVARQKRGIVDQCCTSICSLYQLENYCN

SEQ ID NO: 22 - protein, 84 aa, Mus sp.
FVKQHLCGPHLVEALYLVCGERGFFYTPKSRREVEDPQVEQLELGGSPGDLQTLALEVARQKRGIVDQCCTSICSLYQLENYCN

SEQ ID NO: 23 - protein, 81 aa, Bos sp.
FVNQHLCGSHLVEALYLVCGERGFFYTPKARREVEGPQVGALELAGGPGAGGLEGPPQKRGIVEQCCASVCSLYQLENYCN

SEQ ID NO: 24 - protein, 81 aa, Ovis aries
FVNQHLCGSHLVEALYLVCGERGFFYTPKARREVEGPQVGALELAGGPGAGGLEGPPQKRGIVEQCCAGVCSLYQLENYCN